European Patent Application EP 4 265 738 A1, published October 25, 2023. Title: COMBINATION OF DNA METHYLATION MARKERS AND USE THEREOF, PRIMERS, PROBES AND KIT FOR EARLY DETECTION OF OVARIAN CANCER. Applicant: BEIJING ORIGIN-POLY BIO-TEC CO.,LTD. Application EP22737702.5. The sequence listing filed with the application follows.

SEQUENCE LISTING (51 sequences)

SEQ ID NO: 1 - DNA, 102 bp, Artificial Sequence
  PCDHB18P gene fragment chr5:141235136-141235232
actggaccaatccctggatcgagaaaaggtgtctgagtttagtttaacgctaacagccgtggatggcgggtctccgcccaggtctgggactacactgattaa

SEQ ID NO: 2 - DNA, 123 bp, Artificial Sequence
  PCDHB18P gene fragment chr5:141235796-141235918
aaatgaatataacatcaccatcaccgtgaccgacttggggacacccaggctgaaaaccgagcacaacataaccgtgctggtctccgacgtcaatgacaacgcccccatcttcacccaaacctc

SEQ ID NO: 3 - DNA, 83 bp, Artificial Sequence
  PCDHB18P gene fragment chr5:141235982-141236064
agacagagactcaggcaccaacgcccaggtcacctactcgctgctgccgccccaggacccgcacctgcccctcacctccctgg

SEQ ID NO: 4 - DNA, 100 bp, Artificial Sequence
  CDO1 gene fragment Chr5:115816656-115816755
tcttgggtggctctccgcctcgtcctccctccgagggccgttggtacattcctagtgactccaagcgcttaaaaggggcccgggaggatgaaccccacag

SEQ ID NO: 5 - DNA, 78 bp, Artificial Sequence
  CDO1 gene fragment Chr5:115816502-115816579
gtctcttgctgtctctgcgacgacatccttacgtttcggcactctaatgctgggtttgtgcgtgtgtgtctgcttagc

SEQ ID NO: 6 - DNA, 79 bp, Artificial Sequence
  CDO1 gene fragment Chr5:115816382-115816460
gctcgctcagctcctccaccgcagcccagcagtgagacgcgcgcgcagccagctccccacgagatggaacagaccgaag

SEQ ID NO: 7 - DNA, 93 bp, Artificial Sequence
  HOXA9 gene fragment chr7:27166431-27166523
gccagctgatgagaaaggcgggctgggcgcgcgtgtgcgtggggtcgagggccggggaccgagcgcgccgcacaaccaaccaggccctcaaaa

SEQ ID NO: 8 - DNA, 107 bp, Artificial Sequence
  HOXA9 gene fragment chr7:27166020-27166126
cagtctaacctttccaagtcctcgtaaatttttacagctgggagccacggcgaggcaaacgaatctgttggtcgtttccgacttcccgccagcctgtgtggcttctg

SEQ ID NO: 9 - DNA, 85 bp, Artificial Sequence
  HOXA9 gene fragment chr7:27165835-27165919
tttatgtgaggggctccgctggccgcactcgcacgcgggacccgcgccttcttgatggcgtgattaattgtgatataaaatagtc

SEQ ID NO: 10 - DNA, 107 bp, Artificial Sequence
  LYPD5 gene fragment chr19:43820817-43820923
tgaaatttgataactgaaaacgaagtatgccatctgtttccgttatcagtttattgctctcacctccgcacgcactcttcaatatacgctccctgctaaagggattc

SEQ ID NO: 11 - DNA, 70 bp, Artificial Sequence
  LYPD5 gene fragment chr19:43820625-43820694
ttcccacaggtcactgggccgaatgagcgtgcgctcctgatccgctttgcgcatcccagtgattcttggg

SEQ ID NO: 12 - DNA, 107 bp, Artificial Sequence
  LYPD5 gene fragment chr19:43820271-43820377
ggtgtgtgcaatattatgtgcgtgatagagccaaggatgtgccctaccgtgcgaatggtgacgttgcgtctgtatgagagtgcacgtgccacggctgggatgtcttg

SEQ ID NO: 13 - DNA, 28 bp, Artificial Sequence
  PCDHB18P target gene detection forward primer for chr5:141235136-141235232
atccaaaattggattaatttttggatcg

SEQ ID NO: 14 - DNA, 31 bp, Artificial Sequence
  PCDHB18P target gene detection reverse primer for chr5:141235136-141235232
tttaggttcaatataatcccaaacctaaacg

SEQ ID NO: 15 - DNA, 31 bp, Artificial Sequence
  PCDHB18P gene detection probe for chr5:141235136-141235232
  misc_feature (1)..(1): The probe has FAM at the N-terminus of nucleotide 1
  misc_feature (31)..(31): The probe has BHQ1 at the C-terminus of nucleotide 31
ccgccataacgttaatagtcgtggatggcgg

SEQ ID NO: 16 - DNA, 36 bp, Artificial Sequence
  PCDHB18P target gene detection forward primer for chr5:141235796-141235918
ataataataaaaatgaatataatattattattatcg

SEQ ID NO: 17 - DNA, 34 bp, Artificial Sequence
  PCDHB18P target gene detection reverse primer for chr5:141235796-141235918
tttttattttaaaatttaaataaaaataaaaacg

SEQ ID NO: 18 - DNA, 30 bp, Artificial Sequence
  PCDHB18P gene detection probe for chr5:141235796-141235918
  misc_feature (1)..(1): The probe has FAM at the N-terminus of nucleotide 1
  misc_feature (30)..(30): The probe has BHQ1 at the C-terminus of nucleotide 30
ttaacgaatcgtgttggttttcgacgttaa

SEQ ID NO: 19 - DNA, 31 bp, Artificial Sequence
  PCDHB18P target gene forward detection primer for chr5:141235982-141236064
ttaataccagatagagatttaggtattaacg

SEQ ID NO: 20 - DNA, 32 bp, Artificial Sequence
  PCDHB18P target gene reverse detection primer for chr5:141235982-141236064
tatttgttccaaaaaaataaaaaacaaatacg

SEQ ID NO: 21 - DNA, 28 bp, Artificial Sequence
  PCDHB18P gene detection probe for chr5:141235982-141236064
  misc_feature (1)..(1): The probe has FAM at the N-terminus of nucleotide 1
  misc_feature (28)..(28): The probe has BHQ1 at the C-terminus of nucleotide 28
taaaacgttattcgttgttgtcgtttta

SEQ ID NO: 22 - DNA, 24 bp, Artificial Sequence
  CDO1 target gene detection forward primer for Chr5:115816656-115816755
aaaaaccttttgggtggtttttcg

SEQ ID NO: 23 - DNA, 28 bp, Artificial Sequence
  CDO1 target gene detection reverse primer for Chr5:115816656-115816755
ggaggatgctataaaattcatcctcccg

SEQ ID NO: 24 - DNA, 30 bp, Artificial Sequence
  CDO1 gene detection probe for Chr5:115816656-115816755
  misc_feature (1)..(1): The probe has ROX at the N-terminus of nucleotide 1
  misc_feature (30)..(30): The probe has BHQ2 at the C-terminus of nucleotide 30
aacgacctcgtttttttttcgagggtcgtt

SEQ ID NO: 25 - DNA, 26 bp, Artificial Sequence
  CDO1 target gene detection forward primer for Chr5:115816502-115816579
caaaaacgttttttgttgtttttgcg

SEQ ID NO: 26 - DNA, 25 bp, Artificial Sequence
  CDO1 target gene detection reverse primer for Chr5:115816502-115816579
tgtgtgtgctaaacaaacacacacg

SEQ ID NO: 27 - DNA, 27 bp, Artificial Sequence
  CDO1 gene detection probe for Chr5:115816502-115816579
  misc_feature (1)..(1): The probe has ROX at the N-terminus of nucleotide 1
  misc_feature (27)..(27): The probe has BHQ2 at the C-terminus of nucleotide 27
aaaatactttttacgtttcggtatttt

SEQ ID NO: 28 - DNA, 28 bp, Artificial Sequence
  CDO1 target gene detection forward primer for Chr5:115816382-115816460
ataaaaagttcgtttagtttttttatcg

SEQ ID NO: 29 - DNA, 27 bp, Artificial Sequence
  CDO1 target gene detection reverse primer for Chr5:115816382-115816460
agatggacttcgatctattccatctcg

SEQ ID NO: 30 - DNA, 27 bp, Artificial Sequence
  CDO1 target gene detection probe for Chr5:115816382-115816460
  misc_feature (1)..(1): The probe has ROX at the N-terminus of nucleotide 1
  misc_feature (27)..(27): The probe has BHQ2 at the C-terminus of nucleotide 27
taactacgtgagacgcgcgcgtagtta

SEQ ID NO: 31 - DNA, 28 bp, Artificial Sequence
  HOXA9 target gene detection forward primer for chr7:27166431-27166523
cctttctcgttagttgatgagaaaggcg

SEQ ID NO: 32 - DNA, 33 bp, Artificial Sequence
  HOXA9 target gene detection reverse primer for chr7:27166431-27166523
tataattattttaaaaacctaattaattatacg

SEQ ID NO: 33 - DNA, 26 bp, Artificial Sequence
  HOXA9 gene detection probe for chr7:27166431-27166523
  misc_feature (1)..(1): The probe has CY5 at the N-terminus of nucleotide 1
  misc_feature (26)..(26): The probe has BHQ2 at the C-terminus of nucleotide 26
ccacgcatgggcgcgcgtgtgcgtgg

SEQ ID NO: 34 - DNA, 32 bp, Artificial Sequence
  HOXA9 target gene detection forward primer for chr7:27166020-27166126
aaaacttatagtttaatttttttaagttttcg

SEQ ID NO: 35 - DNA, 29 bp, Artificial Sequence
  HOXA9 target gene detection reverse primer for chr7:27166020-27166126
ttagtttgcaaaaaccacacaaactaacg

SEQ ID NO: 36 - DNA, 29 bp, Artificial Sequence
  HOXA9 gene detection probe for chr7:27166020-27166126
  misc_feature (1)..(1): The probe has CY5 at the N-terminus of nucleotide 1
  misc_feature (29)..(29): The probe has BHQ2 at the C-terminus of nucleotide 29
attcgtttattacggcgaggtaaacgaat

SEQ ID NO: 37 - DNA, 27 bp, Artificial Sequence
  HOXA9 target gene detection forward primer for chr7:27165835-27165919
aaacccctctttatgtgaggggtttcg

SEQ ID NO: 38 - DNA, 36 bp, Artificial Sequence
  HOXA9 target gene detection reverse primer for chr7:27165835-27165919
tgattaattaactattttatatcacaattaatcacg

SEQ ID NO: 39 - DNA, 35 bp, Artificial Sequence
  HOXA9 gene detection probe for chr7:27165835-27165919
  misc_feature (1)..(1): The probe has CY5 at the N-terminus of nucleotide 1
  misc_feature (35)..(35): The probe has BHQ2 at the C-terminus of nucleotide 35
aacgcgaattcgtattcgtacgcgggattcgcgtt

SEQ ID NO: 40 - DNA, 30 bp, Artificial Sequence
  LYPD5 target gene detection forward primer for chr19:43820817-43820923
ttttcaattgaaatttgataattgaaaacg

SEQ ID NO: 41 - DNA, 28 bp, Artificial Sequence
  LYPD5 target gene detection reverse primer for chr19:43820817-43820923
ttttttgaaatccctttaacaaaaaacg

SEQ ID NO: 42 - DNA, 36 bp, Artificial Sequence
  LYPD5 gene detection probe for chr19:43820817-43820923
  misc_feature (1)..(1): The probe has HEX at the N-terminus of nucleotide 1
  misc_feature (36)..(36): The probe has BHQ1 at the C-terminus of nucleotide 36
attaaaaagtttttattttcgtacgtattttttaat

SEQ ID NO: 43 - DNA, 28 bp, Artificial Sequence
  LYPD5 target gene detection forward primer for chr19:43820625-43820694
acccaattttttataggttattgggtcg

SEQ ID NO: 44 - DNA, 29 bp, Artificial Sequence
  LYPD5 target gene detection reverse primer for chr19:43820625-43820694
tattttagcccaaaaatcactaaaatacg

SEQ ID NO: 45 - DNA, 28 bp, Artificial Sequence
  LYPD5 gene detection probe for chr19:43820625-43820694
  misc_feature (1)..(1): The probe has HEX at the N-terminus of nucleotide 1
  misc_feature (28)..(28): The probe has BHQ1 at the C-terminus of nucleotide 28
aacgaatagcgtgcgtttttgattcgtt

SEQ ID NO: 46 - DNA, 30 bp, Artificial Sequence
  LYPD5 target gene detection forward primer for chr19:43820271-43820377
cacataatggtgtgtgtaatattatgtgcg

SEQ ID NO: 47 - DNA, 23 bp, Artificial Sequence
  LYPD5 target gene detection reverse primer for chr19:43820271-43820377
gttgggacaaaacatcccaaccg

SEQ ID NO: 48 - DNA, 31 bp, Artificial Sequence
  LYPD5 gene detection probe for chr19:43820271-43820377
  misc_feature (1)..(1): The probe has HEX at the N-terminus of nucleotide 1
  misc_feature (31)..(31): The probe has BHQ1 at the C-terminus of nucleotide 31
acgcaacgtcgtgcgaatggtgacgttgcgt

SEQ ID NO: 49 - DNA, 20 bp, Artificial Sequence
  GAPDH gene forward primer
aggttaaatatagttgttga

SEQ ID NO: 50 - DNA, 17 bp, Artificial Sequence
  GAPDH gene reverse primer
caacccaaacccccaac

SEQ ID NO: 51 - DNA, 18 bp, Artificial Sequence
  GAPDH gene detection probe
  misc_feature (1)..(1): The probe has Joe at the N-terminus of nucleotide 1
  misc_feature (18)..(18): The probe has BHQ1 at the C-terminus of nucleotide 18
tagttgggggtttgggtt